European Patent Specification EP 2 612 912 B1, published March 5, 2025. Title: A protein having glycoalkaloid synthetase activity and a gene encoding the protein. Applicant: KIRIN HOLDINGS KABUSHIKI KAISHA. The sequence listing filed with the application follows.

SEQUENCE LISTING (19 sequences)

SEQ ID NO: 1 - protein, 487 aa, Solanum tuberosum
MDFYNLALFFIALVIGIFTFYAILMRINGWYYAIKFCSKKYNIPLGYMGLPYFGNTLSYFKSTICGDPNSFLDFFATRFGTGGMYRAYIFGKPTIMVTKPEIIRKVLMDEEYLERGLPNYMKKLIGLTTSIEEDKYFRRLTSPVKSHGLLSDYFDYIDKTVSTTLEKYATTEEPIEFLHKMHRLAFEVFMRLLIGDEVNQEFFDQMFVEITAVISAVHNLPINLPGFPYHKGLKARKVLGGIFQKLIDERREAMKDGKSMPRANIIDMLLSNTNQDYEDNILSDKKIVEILVLFSFAGFEPVALMSVKAIFHLQKHPHFLEKAKEEQEEIVKRRASSNAGLSFDEIRQMTFVSKVINETLRIATDQTVFLRDTSTTFNINGYTIPKGWKFFAVVWNIHMNPDVYVQPKEFNPSRWDDIETKPGIFLPFSMGPKSCPGSNLAKLQISVILHYYLLHYRVEQINPEARCYPPENCLVKFKKLSISSDGN

SEQ ID NO: 2 - DNA, 1461 bp, Solanum tuberosum
atggatttctacaatttagccttattcttcatagctttagtaattgggattttcacattttatgctatattaatgagaattaatggttggtattatgcaatcaaattttgttcaaagaaatataacatccctctaggttatatgggtttgccatattttggcaacacactttcttacttcaaatctaccatttgtggtgatccaaattcattccttgatttctttgctactaggtttgggacaggaggaatgtatagggcatacatatttgggaagccaacaattatggtgacaaagccagaaataattagaaaagttttgatggatgaagaatatcttgaaagaggtttgcctaattatatgaaaaaattaattggattaacaacttcgattgaagaagataaatattttcgtcgattaacatctccagtaaaaagtcatggattattatccgattattttgattatatcgataaaactgtgagcactacattagagaaatacgctactacggaagaacctattgagtttctccataagatgcacaggcttgcatttgaggtgtttatgagacttcttattggtgatgaggttaatcaagaattttttgatcaaatgtttgtggagattactgctgtaattagtgctgttcacaacttgccaattaatctcccaggatttccttatcataagggactcaaggctcgaaaagtactaggagggatatttcaaaaactaatagatgaaagaagagaagccatgaaggatggaaaatcaatgccaagggcaaacataattgatatgttgttatcaaacactaatcaagattatgaagacaatatattgagtgacaagaagatcgttgaaatcctagttttgttttcatttgctggttttgaacctgttgctcttatgtctgtcaaggcaatttttcacttgcaaaagcatccccatttcttggagaaagccaaagaggaacaagaggaaatagtaaagagaagagcatcttcaaatgctggacttagttttgatgagattaggcaaatgacgtttgttagtaaggtaattaatgaaacgttacgtattgctactgatcaaacggtattccttagagacacaagtactacttttaacataaatgggtacaccatacccaaagggtggaagttttttgcagttgtatggaatattcatatgaatcctgatgtttatgttcagcctaaggaatttaatccttcaagatgggatgatattgaaactaagccaggcatttttcttccattttcaatgggccccaaatcatgcccaggatccaatctggccaagcttcaaatttcagtaattcttcattattatcttcttcactacagggttgagcaaattaatccagaggctagatgttatcctcctgaaaattgtcttgtgaaattcaagaagctctcaatctctagtgatggtaac

SEQ ID NO: 3 - protein, 487 aa, Solanum lycopersicum
MDFYNLALFFIALILGIFTFYAILMRINGWYYAIKFCSNKYNIPNGYMGLPYFGNTLSYFKASMCGDPKSFIDFFATRFGEGGMYRAYIFGKPTIMVTKPEIIRKVLMDEEYLERGLPNYMKKLIGLTTSIEEDKYFRRLTAPVKSHGLLSDYFDYIDKTVSSTLEKYATTEEPVEFLHKMHKLTFEVFMRLLIGDEVNQELFDEMFEEITAVISGVHNLPINLPGFAYHKGLKARKVLGEVFKKLIDERREAMKDGKSMPKANIIDMLLSNNNQDYEANMLSDKKIIEILVLFSFAGFEPVALMSVKAIFHLQKHPHFLEKAKEEQEEIVKRRASSNAGLSFDEIRQMTFVSKIINETLRIATDQSVFLRDTSTTFNINGYTIPKGWKFFAVVWNIHMNPDVYVQPKEFNPSRWDDIETKPGIFLPFSMGPKSCPGSNLAKLQISVILHYYLLHYRVEQINPEARCYPPENCLVKFKKLSISSNGN

SEQ ID NO: 4 - DNA, 1461 bp, Solanum lycopersicum
atggatttctacaatttagccttgttcttcatagctttaatacttggaattttcacattttatgccatattaatgagaataaatggttggtattatgcaatcaaattttgttcaaacaaatataacatcccaaatggttatatgggtttgccatattttggtaacacactttcttacttcaaagcttcaatgtgtggtgatccaaaatcattcattgatttctttgctactaggtttggagaaggaggaatgtatagggcatacatatttgggaagccaacaattatggtgacaaagccagaaataattagaaaagttttgatggatgaagagtatcttgaaagaggtttgcctaattatatgaaaaaattaattggattaacaacttcgatagaagaagacaaatattttcgtagattaacagcaccagtaaaaagtcatggattattatctgattatttcgattatatcgataaaactgtgagttctacattagagaaatacgctactacggaagaacctgttgagtttcttcataaaatgcacaagcttacgtttgaggtgtttatgagacttttaattggtgatgaagttaatcaagaattatttgatgaaatgtttgaggagattactgctgtaattagtggtgttcacaatttgccaattaatctcccaggatttgcttatcataagggactcaaggctcgaaaagtactaggagaggtatttaaaaaattaattgatgaaagaagagaagccatgaaggatggaaaatcaatgccaaaggcaaacataattgatatgttgttatcaaacaacaatcaagattatgaagcaaacatgttgagtgacaagaagatcattgaaatcctagttttgttttcatttgctggttttgaacctgttgctcttatgtctgtcaaggcaattttccacttacaaaaacatccacatttcttggaaaaagccaaagaggaacaagaggaaatagtaaagagaagagcatcttcaaatgctggacttagttttgatgaaattagacaaatgacatttgttagtaagataattaatgaaacgttacgtatagctactgatcagtcggtattccttagagacacaagtactacttttaacataaatgggtacaccatacccaaagggtggaagttttttgcagttgtatggaatattcatatgaatcctgatgtttatgttcaacctaaggaatttaatccttcgagatgggatgatattgaaactaagccaggcatttttctacctttttcaatgggccccaaatcatgcccaggatccaatttggccaagcttcaaatttcagtaattcttcattattatcttcttcactacagggttgagcaaattaatccagaggctagatgttatcctcctgaaaattgtcttgtgaaattcaagaagctatcgatctctagtaatggtaat

SEQ ID NO: 5 - DNA, 5439 bp, Solanum tuberosum
gaggctaagaaaaagagagagagagaacatggatttctacaatttagccttattcttcatagctttagtaattgggattttcacattttatgctatattaatgagaattaatggttggtattatgcaatcaaattttgttcaaagaaatataacatccctctaggttatatgggtttgccatattttggcaacacactttcttacttcaaatctaccatttgtggtgatccaaattcattccttgatttctttgctactaggtaaattaactattttcattatcgtacttatttgctatgttgtttgaattcttgaaaaatattaatatgtacttgtcaaatcttttaaaaatagtgcatttttgaagaatctaacatgagtactgcaactgttattacaattacatttttgtagagtccaattgaacaaaatttttcttttttttttttaaaggtttgggacaggaggaatgtatagggcatacatatttgggaagccaacaattatggtgacaaagccagaaataattagaaaagttttgatggatgaagaatatcttgaaagaggtttgcctaattatatgaaaaaattaattggattaacaacttcgattgaagaagataaatattttcgtcgattaacatctccagtaaaaagtcatggattattatccgattattttgattatatcgataaaactgtgagcactacattagagaaatacgctactacggaagaacctattgagtttctccataagatgcacaggcttgcatttgaggtgtttatgagacttcttattggtgatgaggttaatcaagaattttttgatcaaatgtttgtggagattactgctgtaattagtgctgttcacaacttgccaattaatctcccaggatttccttatcataagggactcaaggtaagatgtgttcaaacttttaatattatttttatttcattttaaatttttaataatcataagatataaatgtgtttttttaacttgccatcagtttatatttgtgcccttcaattttgagtgtgtataaatttgaattagtagacacatgacataatatatgtaggacatcatgtaggatgcaaactgtcacgaagaacgtgtgtgtttacttgttcaactttatataagtttaagtgtctacttgtgtgtgtccaaaattgaagggtacacatgtgagatgaggccaagttaaatggcatatttatatattttagatagaataacatgtttttttttatatacataatatataaatctgcccttcgatttggattcaactgacatctatgccctccaactttaggtgtgcacaaacatatgcttaaacatgtataaaaatgaacaaatagacacatttgtcttaactggcacacatgacaattttgtgtcctacgtgatgccctacatgtattatgttacgcaggacatgtgtgtcaacttgtttaattttatacaagtttaagtgtctatttgtacacacccaaaattagttgaagccaagttaaatgacatatttatgtattatatattttctacatacataattacatgtgtgggagccccaaccacctcttttatttttttaataattggtgatggtggtgattagagagactagaattaaagatatttgttctgttgtaataccattattgaattgtacggctacttcatttaaggaactattgatttaatttaagtgcaacactcttttcacaaatcaagaactacgaagggtgtgtttggtatgaaaggaaaacattttccagaaaatgcttttcaattttctcatgtttggttgggtaaaatgttttggaaatgttttccaaatcaacttattttcctcaaatttaaggaaaatgacttcccctcaaaaattaagaaaaacattttccaaaactctcctacaactttaaattacaatttatattttttgaaaaaatcaattttttttgttgaaaaaaaaattaaagcttttttttaaaaaaaaaaaatcgacttcaatttttaattttttttatcccaccctcaccccctactccctaccccgccaaatccccttccaccccacaaaaaaaattaagtttttttttaaaaaatgtttccaatttaaattttattttttcatcccaccccctcccttaccctcgacctcctccccaccatcccccctacacccaaaaaattcaaaaaataaagttggttctaaaatatatttctaattcaaattcttatttttcatccacccaccccccggccagcccacccccaccaaaaaaaattaagtttgtttttaaaaaaatattttttatttcaaatttttatttttccaccccaccccctacccgcgaccccccatcagccccccaccccctccaaaaaaaaatttaagtttattttaaaaaaaatattttcaatttcattttttgttttttcaccccaccccctacccgccagcctcaccccccaaccccaccctcccccaaaaaaatttaagtttattttaaaaaaaatattttcagtttcaattcaaaaaattattctctctagttagaataaaagatattttctcaaaaaaaaaaatcattcataaatcaaacacataaaaatctttttcgaaaaatattttatactcaccaaccaaacatgagaaaataagtccaaagtctacttattttccaggaaaacattttccttcataccgaacacacccgaaatcacccctttcatcttttatcgtgatatttgtggttgtaataaacataatatagagtgcaacatgcatgtcaaagaccaaaaactatgagatcactcttttcatttaatatttatcgtgttgtatatgtttattatgatttcaggctcgaaaagtactaggagggatatttcaaaaactaatagatgaaagaagagagaagcctgaaggatggaaaatcaatgccaagggcaaacataattgatgtgttgttatcaaacactaatcaagattatgaagacaatatattgagtgacaagaagatcgttgaaatcctagttttgttttcatttgctggttttgaacctgttgctcttatgtctgtcaaggcaatttttcacttgcaaaagcatccccatttcttggagaaagccaaagtaagtactctttattctgttttaggggtgtcatatgggtgagttaaactgaatttggacaggtggactgagttaattagtccaaaacttacttggactaaaatggactaacaaacgagtcataaactcaactcgtctaattagacaggttgagttaaatttggacgaattaaattgggctaagttaatatgtccaaaaatttggggctaaaatgagataacaaaaggatcataactcaactcgtctaattggtcgatccaaacctaagcgggttgggtgggtagtgtattcacgagtggatttgccacccctagtttattttattttatatgacgatatttgattaattatttttttaacaggaggaacaagaggaaatagtaaagagaagagcatcttcaaatgctggacttagttttgatgagattaggcaaatgacgtttgttagtaaggtaagacaatattatgatgttatatactttctataatagcatttttataaataataccattatacaaaaagtcatcagtacaaataattaaaaaaagaagatgaagtgataatacaaaaattggactaacatgcattattatttattaatgttatctcttttaatattgacaggtaattaatgaaacgttacgtattgctactgatcaaacggtattccttagagacacaagtactacttttaacataaatggttggtactttgccttattcttttgtatttatattattattttctatcgaaaaatcaaaatacgacaaatattttgaaacgacgaataattcattcattcatttatctcttgtatgtgtagggtacaccatacccaaagggtggaagttttttgcagttgtatggaatattcatatgaatcctgatgtttatgttcagcctaaggaatttaatccttcaagatgggatgtaagtgatatgcatcttaattaattgtgtttaagaaaaaaattcactttattttttttataatcaagaaatttttgagggttaataatgtatgattcaaaatatgttacgtaataagttgtgtttgccttttaccactttgaatattaggtattttatttgcagtagggtttaaactcatgacgagaatttatttatacataagaatattagtaaaattagctcataaaaatatgatttgttcaatgtcttatttattaattcaattaattttgactcatctaatttaattcatctaaaaaatagtgctaggataataataataataataataaaatcggaaatgtgctctaaactagaaccacgccctccactaggaagaaaaaaaattgattaacaatctcttaacattcttcaaacctaattttgaacctcggtatgttctcctattttgagttatagcctcgatgagttaaagacgaatcatgtcatatctagctaatcaattcttttcaaatcttcctcgatctatctctacctctccttaaacatcgttgtcaatcttttgtaccttaggagtaaaagataggatattagttgctttaccgttctcaatggtacatagctaaaaagtgtattatcatcaggacaatgcatgtgttcctccttttgagatatctgaactatctcaatttaactttttacgttacgaaaatcattcccacattacttattacttaatgatcaagtgaaatttgacaggatattgaaactaagccaggcatttttcttccattttcaatgggccccaaatcatgcccaggatccaatctggccaagcttcaaatttcagtaattcttcattattatcttcttcactacaggtaattaaatagcttcatacttataatatgaaaaaattaactaattatattttgaatattttattttattttcttaccaaatattttcaaagggactaaaatatatgaatttattgtgaaatttataccaaaaaataagtattttgacccttatactcgtgattttatcgtatgaattgagatggatggaatatttaaaataaaaaaggaaatataaattattgattaaatcatattttaatttaattaaacgatatatttaatattcatgcagggttgagcaaattaatccagaggctagatgttatcctcctgaaaattgtcttgtgaaattcaagaagctctcaatctctagtgatggtaactaattttaatcattgtgctacaaataaataattcatgttgtaatcttgaaaacaataagtgtattgaataattattaaattggatgtttttgtagaacg

SEQ ID NO: 6 - DNA, 24 bp, Artificial
  primer
gaggctaagaaaaagagagagaga

SEQ ID NO: 7 - DNA, 23 bp, Artificial
  primer
cgttctacaaaaacatccaattt

SEQ ID NO: 8 - DNA, 21 bp, Artificial
  primer
tgataaggaaatcctgggaga

SEQ ID NO: 9 - DNA, 20 bp, Artificial
  primer
agagaagccatgaaggatgg

SEQ ID NO: 10 - DNA, 24 bp, Artificial
  primer
gaaatacgctactacggaagaacc

SEQ ID NO: 11 - DNA, 21 bp, Artificial
  primer
cgtcatttgcctaatctcatc

SEQ ID NO: 12 - DNA, 29 bp, Artificial
  primer
gagctctagaggtttgggacaggaggaat

SEQ ID NO: 13 - DNA, 29 bp, Artificial
  primer
ggatccatatgcaagcctgtgcatcttat

SEQ ID NO: 14 - DNA, 19 bp, Artificial
  primer
taaagcacgaggaagcggt

SEQ ID NO: 15 - DNA, 19 bp, Artificial
  primer
gcacaacagacaatcggct

SEQ ID NO: 16 - DNA, 20 bp, Artificial
  primer
taagggactcaaggctcgaa

SEQ ID NO: 17 - DNA, 20 bp, Artificial
  primer
ttcctctttggctttctcca

SEQ ID NO: 18 - DNA, 19 bp, Artificial
  primer
taaagcacgaggaagcggt

SEQ ID NO: 19 - DNA, 19 bp, Artificial
  primer
gcacaacagacaatcggct